European Patent Specification EP 4 101 864 B1, published October 22, 2025. Title: Polypeptide, preparation method and use thereof. Applicant: Fudan University SHANXI JINBO BIO-PHARMACEUTICAL CO., LTD. The sequence listing filed with the application follows.

SEQUENCE LISTING (5 sequences)

SEQ ID NO: 1 - protein, 36 aa, artificial sequence
  2019-HR2P
DISGINASVVNIQKEIDRLNEVAKNLNESLIDLQEL

SEQ ID NO: 2 - protein, 36 aa, artificial sequence
  EK1
SLDQINVTFLDLEYEMKKLEEAIKKLEESYIDLKEL

SEQ ID NO: 3 - protein, 42 aa, artificial sequence
  2019-HR1P
ANQFNSAIGKIQDSLSSTASALGKLQDVVNQNAQALNTLVKQ

SEQ ID NO: 4 - protein, 1295 aa, Coronavirus
MPMGSLQPLATLYLLGMLVASVLAQCVNLTTRTQLPPAYTNSFTRGVYYPDKVFRSSVLHSTQDLFLPFFSNVTWFHAIHVSGTNGTKRFDNPVLPFNDGVYFASTEKSNIIRGWIFGTTLDSKTQSLLIVNNATNVVIKVCEFQFCNDPFLGVYYHKNNKSWMESEFRVYSSANNCTFEYVSQPFLMDLEGKQGNFKNLREFVFKNIDGYFKIYSKHTPINLVRDLPQGFSALEPLVDLPIGINITRFQTLLALHRSYLTPGDSSSGWTAGAAAYYVGYLQPRTFLLKYNENGTITDAVDCALDPLSETKCTLKSFTVEKGIYQTSNFRVQPTESIVRFPNITNLCPFGEVFNATRFASVYAWNRKRISNCVADYSVLYNSASFSTFKCYGVSPTKLNDLCFTNVYADSFVIRGDEVRQIAPGQTGKIADYNYKLPDDFTGCVIAWNSNNLDSKVGGNYNYLYRLFRKSNLKPFERDISTEIYQAGSTPCNGVEGFNCYFPLQSYGFQPTNGVGYQPYRVVVLSFELLHAPATVCGPKKSTNLVKNKCVNFNFNGLTGTGVLTESNKKFLPFQQFGRDIADTTDAVRDPQTLEILDITPCSFGGVSVITPGTNTSNQVAVLYQDVNCTEVPVAIHADQLTPTWRVYSTGSNVFQTRAGCLIGAEHVNNSYECDIPIGAGICASYQTQTNSPRRARSVASQSIIAYTMSLGAENSVAYSNNSIAIPTNFTISVTTEILPVSMTKTSVDCTMYICGDSTECSNLLLQYGSFCTQLNRALTGIAVEQDKNTQEVFAQVKQIYKTPPIKDFGGFNFSQILPDPSKPSKRSFIEDLLFNKVTLADAGFIKQYGDCLGDIAARDLICAQKFNGLTVLPPLLTDEMIAQYTSALLAGTITSGWTFGAGAALQIPFAMQMAYRFNGIGVTQNVLYENQKLIANQFNSAIGKIQDSLSSTASALGKLQDVVNQNAQALNTLVKQLSSNFGAISSVLNDILSRLDKVEAEVQIDRLITGRLQSLQTYVTQQLIRAAEIRASANLAATKMSECVLGQSKRVDFCGKGYHLMSFPQSAPHGVVFLHVTYVPAQEKNFTTAPAICHDGKAHFPREGVFVSNGTHWFVTQRNFYEPQIITTDNTFVSGNCDVVIGIVNNTVYDPLQPELDSFKEELDKYFKNHTSPDVDLGDISGINASVVNIQKEIDRLNEVAKNLNESLIDLQELGKYEQYIKWPWYIWLGFIAGLIAIVMVTIMLCCMTSCCSCLKGCCSCGSCCKFDEDDSEPVLKGVKLHYTGGTETSQVAPA

SEQ ID NO: 5 - DNA, 3906 bp, Coronavirus
ggatccgccaccatgcccatggggtctctgcaaccgctggccaccttgtacctgctggggatgctggtcgcttccgtgctagcccagtgcgtgaacctgaccacaaggacccagctgccccctgcctataccaattccttcacacggggcgtgtactatcccgacaaggtgtttagaagctccgtgctgcactctacacaggatctgtttctgcctttctttagcaacgtgacctggttccacgccatccacgtgagcggcaccaatggcacaaagcggttcgacaatccagtgctgccctttaacgatggcgtgtacttcgcctctaccgagaagagcaacatcatcagaggctggatctttggcaccacactggactccaagacacagtctctgctgatcgtgaacaatgccaccaacgtcgtgatcaaggtgtgcgagttccagttttgtaatgatcctttcctgggcgtgtactatcacaagaacaataagagctggatggagtccgagtttcgcgtgtattctagcgccaacaattgcacatttgagtacgtgtcccagccattcctgatggacctggagggcaagcagggcaatttcaagaacctgagggagttcgtgtttaagaatatcgatggctacttcaagatctactctaagcacaccccaatcaacctggtgcgcgacctgccacagggcttcagcgccctggagccactggtggatctgcccatcggcatcaacatcacccggtttcagacactgctggccctgcacagaagctacctgacacctggcgactcctctagcggatggaccgcaggagctgccgcctactatgtgggctatctgcagccaaggaccttcctgctgaagtacaacgagaatggcaccatcacagacgcagtggattgcgcactggaccccctgagcgagaccaagtgtacactgaagtcctttaccgtggagaagggcatctatcagacatccaatttcagggtgcagcccaccgagtctatcgtgcgctttcccaatatcacaaacctgtgcccttttggcgaggtgttcaacgcaaccaggttcgcaagcgtgtacgcatggaataggaagcggatcagcaactgcgtggccgactatagcgtgctgtacaactccgcctctttcagcacctttaagtgctatggcgtgtcccccacaaagctgaatgacctgtgctttaccaacgtgtacgccgattctttcgtgatcaggggcgacgaggtgcgccagatcgcaccaggacagacaggcaagatcgcagactacaattataagctgcctgacgatttcaccggctgcgtgatcgcctggaacagcaacaatctggattccaaagtgggcggcaactacaattatctgtaccggctgtttagaaagtctaatctgaagccattcgagagggacatctctacagagatctaccaggcaggcagcaccccatgcaatggagtggagggctttaactgttatttccctctgcagagctacggcttccagccaacaaacggcgtgggctatcagccctaccgcgtggtggtgctgagctttgagctgctgcacgcacctgcaacagtgtgcggaccaaagaagtccaccaatctggtgaagaacaagtgcgtgaacttcaacttcaacggactgaccggcacaggcgtgctgaccgagtccaacaagaagttcctgccctttcagcagttcggcagggacatcgcagataccacagacgccgtgcgcgaccctcagaccctggagatcctggacatcacaccatgctctttcggcggcgtgagcgtgatcacacctggcaccaatacaagcaaccaggtggccgtgctgtatcaggacgtgaattgtaccgaggtgcccgtggcaatccacgcagatcagctgacccctacatggcgggtgtacagcaccggctccaacgtgttccagacaagagccggatgcctgatcggagcagagcacgtgaacaattcctatgagtgcgacatccctatcggcgccggcatctgtgcctcttaccagacccagacaaactctccaaggagagcccggagcgtggcatcccagtctatcatcgcctatacaatgagcctgggcgccgagaacagcgtggcctactctaacaatagcatcgccatccctaccaacttcacaatctccgtgaccacagagatcctgccagtgtccatgaccaagacatctgtggactgcacaatgtatatctgtggcgattctaccgagtgcagcaacctgctgctgcagtacggcagcttttgtacccagctgaatagagccctgacaggcatcgccgtggagcaggacaagaacacacaggaggtgttcgcccaggtgaagcagatctacaagaccccacccatcaaggactttggcggcttcaatttttcccagatcctgcccgatccttccaagccttctaagcggagctttatcgaggacctgctgttcaacaaggtgaccctggccgatgccggcttcatcaagcagtatggcgattgcctgggcgacatcgccgccagagacctgatctgtgcccagaagtttaatggcctgaccgtgctgcctccactgctgacagatgagatgatcgcacagtacacaagcgccctgctggcaggcaccatcacatccggatggaccttcggcgcaggagccgccctgcagatccccttcgctatgcagatggcctatcggttcaacggcatcggcgtgacccagaatgtgctgtacgagaaccagaagctgatcgccaatcagtttaactccgccatcggcaagatccaggacagcctgtcctctacagcctccgccctgggcaagctgcaggatgtggtgaatcagaacgcccaggccctgaataccctggtgaagcagctgagctccaacttcggcgccatctctagcgtgctgaatgacatcctgagccggctggacaaggtggaggcagaggtgcagatcgaccggctgatcacaggcagactgcagtctctgcagacctacgtgacacagcagctgatcagggcagcagagatcagggcaagcgccaatctggcagcaaccaagatgtccgagtgcgtgctgggccagtctaagagagtggacttttgtggcaagggctatcacctgatgtccttcccacagtctgcccctcacggagtggtgtttctgcacgtgacctacgtgccagcccaggagaagaacttcaccacagcaccagcaatctgccacgatggcaaggcacactttcccagggagggcgtgttcgtgagcaacggcacccactggtttgtgacacagcgcaatttctacgagcctcagatcatcaccacagacaatacattcgtgtccggcaactgtgacgtggtcatcggcatcgtgaacaataccgtgtatgatcctctgcagccagagctggacagctttaaggaggagctggataagtacttcaagaatcacacctccccagacgtggatctgggcgacatcagcggcatcaatgcctccgtggtgaacatccagaaggagatcgacaggctgaacgaggtggccaagaatctgaacgagagcctgatcgatctgcaggagctgggcaagtatgagcagtacatcaagtggccctggtatatctggctgggcttcatcgccggcctgatcgctatcgtgatggtgaccatcatgctgtgctgtatgacatcctgctgttcttgcctgaagggctgctgtagctgtggctcctgctgtaagtttgatgaggacgattccgagccagtgctgaagggcgtgaagctgcactacaccggcggcaccgagacatctcaggtggcccccgcctaactcgag